European Patent Application EP 4 585 678 A1, published July 16, 2025. Title: 长双歧杆菌婴儿亚种、微生物菌剂及其应用. Applicant: 广州集妍化妆品科技有限公司. The sequence listing filed with the application follows.

SEQUENCE LISTING (89 sequences)

SEQ ID NO: 1 - DNA, 20 bp, synthetic construct
  source 1..20: mol_type = other DNA
agagtttgatcmtggctcag

SEQ ID NO: 2 - DNA, 19 bp, synthetic construct
  source 1..19: mol_type = other DNA
ggttaccttgttacgactt

SEQ ID NO: 3 - DNA, 1354 bp, synthetic construct
  source 1..1354: mol_type = other DNA
tgcaagtcgaacgggatccatcaggctttgcttggtggtgagagtggcgaacgggtgagtaatgcgtgaccgacctgccccatacaccggaatagctcctggaaacgggtggtaatgccggatgttccagttgatcgcatggtcttctgggaaagctttcgcggtatgggatggggtcgcgtcctatcagcttgacggcggggtaacggcccaccgtggcttcgacgggtagccggcctgagagggcgaccggccacattgggactgagatacggcccagactcctacgggaggcagcagtggggaatattgcacaatgggcgcaagcctgatgcagcgacgccgcgtgagggatggaggccttcgggttgtaaacctcttttatcggggagcaagcgtgagtgagtttacccgttgaataagcaccggctaactacgtgccagcagccgcggtaatacgtagggtgcaagcgttatccggaattattgggcgtaaagggctcgtaggcggttcgtcgcgtccggtgtgaaagtccatcgcttaacggtggatccgcgccgggtacgggcgggcttgagtgcggtaggggagactggaattcccggtgtaacggtggaatgtgtagatatcgggaagaacaccaatggcgaaggcaggtctctgggccgttactgacgctgaggagcgaaagcgtggggagcgaacaggattagataccctggtagtccacgccgtaaacggtggatgctggatgtggggcccgttccacgggttccgtgtcggagctaacgcgttaagcatcccgcctggggagtacggccgcaaggctaaaactcaaagaaattgacgggggtccgcacaagcggcggagcatgcggattaattcgatgcaacgcgaagaaccttacctgggcttgacatgttcccgacgatcccagagatggggtttcccttcggggcgggttcacaggtggtgcatggtcgtcgtcagctcgtgtcgtgagatgttgggttaagtcccgcaacgagcgcaaccctcgccccgtgttgccagcggattgtgccgggaactcacgggggaccgccggggttaactcggaggaaggtggggatgacgtcagatcatcatgccccttacgtccagggcttcacgcatgctacaatggccggtacaacgggatgcgacgcggcgacgcggagcggatccctgaaaaccggtctcagttcggatcgcagtctgcaactcgactgcgtgaaggcggagtcgctagtaatcgcgaatcagcaacgtcgcggtgaatgcgttcccgggccttgtacacaccgcccgtcaagtcatgaaagtgggcagca

SEQ ID NO: 4 - DNA, 20 bp, synthetic construct
  source 1..20: mol_type = other DNA
agggaagatccaagagccca

SEQ ID NO: 5 - DNA, 20 bp, synthetic construct
  source 1..20: mol_type = other DNA
actctggatcccctacgctt

SEQ ID NO: 6 - DNA, 20 bp, synthetic construct
  source 1..20: mol_type = other DNA
cttggaacatggcctagctc

SEQ ID NO: 7 - DNA, 20 bp, synthetic construct
  source 1..20: mol_type = other DNA
cattcccagcacaacagaga

SEQ ID NO: 8 - DNA, 20 bp, synthetic construct
  source 1..20: mol_type = other DNA
aaagaagagcaggtgctgga

SEQ ID NO: 9 - DNA, 20 bp, synthetic construct
  source 1..20: mol_type = other DNA
tgctcactggtgttctggag

SEQ ID NO: 10 - DNA, 20 bp, synthetic construct
  source 1..20: mol_type = other DNA
cagcctcccttatcgtgtgt

SEQ ID NO: 11 - DNA, 20 bp, synthetic construct
  source 1..20: mol_type = other DNA
caagggctgtaaaaaggcgg

SEQ ID NO: 12 - DNA, 21 bp, synthetic construct
  source 1..21: mol_type = other DNA
gcgagctaagcccaaggtgta

SEQ ID NO: 13 - DNA, 25 bp, synthetic construct
  source 1..25: mol_type = other DNA
gatgaccatcacaatctcatctcca

SEQ ID NO: 14 - DNA, 23 bp, synthetic construct
  source 1..23: mol_type = other DNA
tcctcatcatgggattcttggtc

SEQ ID NO: 15 - DNA, 21 bp, synthetic construct
  source 1..21: mol_type = other DNA
gaacattcgggaacaggctca

SEQ ID NO: 16 - DNA, 20 bp, synthetic construct
  source 1..20: mol_type = other DNA
tctcctctgttccgggtagg

SEQ ID NO: 17 - DNA, 20 bp, synthetic construct
  source 1..20: mol_type = other DNA
cgtccatccactctgcactt

SEQ ID NO: 18 - DNA, 25 bp, synthetic construct
  source 1..25: mol_type = other DNA
gctggaaaccaacaagactgcttta

SEQ ID NO: 19 - DNA, 25 bp, synthetic construct
  source 1..25: mol_type = other DNA
tatagtggaaccttggctgctggta

SEQ ID NO: 20 - DNA, 21 bp, synthetic construct
  source 1..21: mol_type = other DNA
agtgaggatggcagctctgga

SEQ ID NO: 21 - DNA, 22 bp, synthetic construct
  source 1..22: mol_type = other DNA
atgagatgtgggcagcatgaac

SEQ ID NO: 22 - DNA, 20 bp, synthetic construct
  source 1..20: mol_type = other DNA
gcctggctcgaaacatctga

SEQ ID NO: 23 - DNA, 23 bp, synthetic construct
  source 1..23: mol_type = other DNA
ctgacctggactggaaacggata

SEQ ID NO: 24 - DNA, 25 bp, synthetic construct
  source 1..25: mol_type = other DNA
gcatgaagtgtatgaagtgcttgga

SEQ ID NO: 25 - DNA, 23 bp, synthetic construct
  source 1..23: mol_type = other DNA
ccataccatgctgtggcaactaa

SEQ ID NO: 26 - DNA, 25 bp, synthetic construct
  source 1..25: mol_type = other DNA
tttggctaggtatcattcaactctc

SEQ ID NO: 27 - DNA, 22 bp, synthetic construct
  source 1..22: mol_type = other DNA
cccttagggcaggtagattcag

SEQ ID NO: 28 - DNA, 20 bp, synthetic construct
  source 1..20: mol_type = other DNA
atagccttcgacccaagcaa

SEQ ID NO: 29 - DNA, 21 bp, synthetic construct
  source 1..21: mol_type = other DNA
gagcacggtagggacagttca

SEQ ID NO: 30 - DNA, 18 bp, synthetic construct
  source 1..18: mol_type = other DNA
tgcggtgggaacaagaaa

SEQ ID NO: 31 - DNA, 23 bp, synthetic construct
  source 1..23: mol_type = other DNA
gacaatctgccaagaggagaaga

SEQ ID NO: 32 - DNA, 20 bp, synthetic construct
  source 1..20: mol_type = other DNA
gaatggaacggtgtgtggac

SEQ ID NO: 33 - DNA, 23 bp, synthetic construct
  source 1..23: mol_type = other DNA
cccctttctccttttcttcactt

SEQ ID NO: 34 - DNA, 20 bp, synthetic construct
  source 1..20: mol_type = other DNA
gtgagcgaggagcttgatgt

SEQ ID NO: 35 - DNA, 20 bp, synthetic construct
  source 1..20: mol_type = other DNA
tcatccttgggttggatggc

SEQ ID NO: 36 - DNA, 20 bp, synthetic construct
  source 1..20: mol_type = other DNA
cagcgaccagacagatgagg

SEQ ID NO: 37 - DNA, 20 bp, synthetic construct
  source 1..20: mol_type = other DNA
gaccttgaggctgagtggag

SEQ ID NO: 38 - DNA, 20 bp, synthetic construct
  source 1..20: mol_type = other DNA
ctgaaggttctgatgccagc

SEQ ID NO: 39 - DNA, 20 bp, synthetic construct
  source 1..20: mol_type = other DNA
taggtctccatgggttggga

SEQ ID NO: 40 - DNA, 21 bp, synthetic construct
  source 1..21: mol_type = other DNA
cctcaatggggctactgttgt

SEQ ID NO: 41 - DNA, 20 bp, synthetic construct
  source 1..20: mol_type = other DNA
gcccatcaatgaagtcggca

SEQ ID NO: 42 - DNA, 24 bp, synthetic construct
  source 1..24: mol_type = other DNA
aattgtccatctgcctctgagtag

SEQ ID NO: 43 - DNA, 23 bp, synthetic construct
  source 1..23: mol_type = other DNA
gtatgaccaggttgcttgtatgc

SEQ ID NO: 44 - DNA, 19 bp, synthetic construct
  source 1..19: mol_type = other DNA
gtgccactgttgaggcttt

SEQ ID NO: 45 - DNA, 20 bp, synthetic construct
  source 1..20: mol_type = other DNA
atggggatactgagggctgt

SEQ ID NO: 46 - DNA, 25 bp, synthetic construct
  source 1..25: mol_type = other DNA
aggatatacacccctaatggagaca

SEQ ID NO: 47 - DNA, 22 bp, synthetic construct
  source 1..22: mol_type = other DNA
aagcaagcaaagcggaaactac

SEQ ID NO: 48 - DNA, 19 bp, synthetic construct
  source 1..19: mol_type = other DNA
aacagcagtgcagatgacg

SEQ ID NO: 49 - DNA, 20 bp, synthetic construct
  source 1..20: mol_type = other DNA
cggttgacccttcaggtgtt

SEQ ID NO: 50 - DNA, 20 bp, synthetic construct
  source 1..20: mol_type = other DNA
ggggactccgtaaaacaggg

SEQ ID NO: 51 - DNA, 20 bp, synthetic construct
  source 1..20: mol_type = other DNA
tcctcgtgcacgcttaagtt

SEQ ID NO: 52 - DNA, 23 bp, synthetic construct
  source 1..23: mol_type = other DNA
attacgaccgctgagttatccac

SEQ ID NO: 53 - DNA, 21 bp, synthetic construct
  source 1..21: mol_type = other DNA
tcaggcacccacttttctttc

SEQ ID NO: 54 - DNA, 20 bp, synthetic construct
  source 1..20: mol_type = other DNA
gtggcagtgatggaagtgtg

SEQ ID NO: 55 - DNA, 20 bp, synthetic construct
  source 1..20: mol_type = other DNA
aggaccagcgttaccaacag

SEQ ID NO: 56 - DNA, 20 bp, synthetic construct
  source 1..20: mol_type = other DNA
accaggagctaacggtctca

SEQ ID NO: 57 - DNA, 20 bp, synthetic construct
  source 1..20: mol_type = other DNA
tctgatccagggtttccatc

SEQ ID NO: 58 - DNA, 20 bp, synthetic construct
  source 1..20: mol_type = other DNA
aggtgtcattgggtttcctg

SEQ ID NO: 59 - DNA, 21 bp, synthetic construct
  source 1..21: mol_type = other DNA
ggtcctcttgtcccttttgtt

SEQ ID NO: 60 - DNA, 20 bp, synthetic construct
  source 1..20: mol_type = other DNA
actgtgattgccctctacgc

SEQ ID NO: 61 - DNA, 20 bp, synthetic construct
  source 1..20: mol_type = other DNA
ggctgtggtattctggatgg

SEQ ID NO: 62 - DNA, 23 bp, synthetic construct
  source 1..23: mol_type = other DNA
gtgtgcttgacagtgttctagtg

SEQ ID NO: 63 - DNA, 22 bp, synthetic construct
  source 1..22: mol_type = other DNA
agttctgcttgacattcctcca

SEQ ID NO: 64 - DNA, 23 bp, synthetic construct
  source 1..23: mol_type = other DNA
gtgtgggcatttcttcctgttag

SEQ ID NO: 65 - DNA, 24 bp, synthetic construct
  source 1..24: mol_type = other DNA
tcaaagtcatcttcagcagtcact

SEQ ID NO: 66 - DNA, 19 bp, synthetic construct
  source 1..19: mol_type = other DNA
accatcaaccgccagagtc

SEQ ID NO: 67 - DNA, 18 bp, synthetic construct
  source 1..18: mol_type = other DNA
gacagccaccgacctcag

SEQ ID NO: 68 - DNA, 20 bp, synthetic construct
  source 1..20: mol_type = other DNA
tccaggtgtaggtggagctt

SEQ ID NO: 69 - DNA, 20 bp, synthetic construct
  source 1..20: mol_type = other DNA
gtgtagggcagtccatagcc

SEQ ID NO: 70 - DNA, 20 bp, synthetic construct
  source 1..20: mol_type = other DNA
agccagtcgaggatacctgt

SEQ ID NO: 71 - DNA, 20 bp, synthetic construct
  source 1..20: mol_type = other DNA
gcaccaaagcctgaaaccag

SEQ ID NO: 72 - DNA, 20 bp, synthetic construct
  source 1..20: mol_type = other DNA
actcggacacaaggttggac

SEQ ID NO: 73 - DNA, 20 bp, synthetic construct
  source 1..20: mol_type = other DNA
ttaggaagctgacccaggag

SEQ ID NO: 74 - DNA, 20 bp, synthetic construct
  source 1..20: mol_type = other DNA
ggtgcggctcatgtttacag

SEQ ID NO: 75 - DNA, 20 bp, synthetic construct
  source 1..20: mol_type = other DNA
gatggcgtctgataccacgg

SEQ ID NO: 76 - DNA, 25 bp, synthetic construct
  source 1..25: mol_type = other DNA
tctctgtgttaggggtatatgatgg

SEQ ID NO: 77 - DNA, 19 bp, synthetic construct
  source 1..19: mol_type = other DNA
gaaggtcgctggacgattt

SEQ ID NO: 78 - DNA, 21 bp, synthetic construct
  source 1..21: mol_type = other DNA
ctctgagaaacctcgggaaac

SEQ ID NO: 79 - DNA, 20 bp, synthetic construct
  source 1..20: mol_type = other DNA
atgaaaactacgaaagcggg

SEQ ID NO: 80 - DNA, 21 bp, synthetic construct
  source 1..21: mol_type = other DNA
acaactgccaaatgggcttga

SEQ ID NO: 81 - DNA, 25 bp, synthetic construct
  source 1..25: mol_type = other DNA
ctgtccctgaacagcccagtactta

SEQ ID NO: 82 - DNA, 20 bp, synthetic construct
  source 1..20: mol_type = other DNA
caggctttcccaagcaaata

SEQ ID NO: 83 - DNA, 20 bp, synthetic construct
  source 1..20: mol_type = other DNA
tgggtcaaactccaactgtg

SEQ ID NO: 84 - DNA, 20 bp, synthetic construct
  source 1..20: mol_type = other DNA
ctgttgttgctgtggctgat

SEQ ID NO: 85 - DNA, 21 bp, synthetic construct
  source 1..21: mol_type = other DNA
tctggttgacttctggtgtcc

SEQ ID NO: 86 - DNA, 21 bp, synthetic construct
  source 1..21: mol_type = other DNA
gcagggaccaggaaaaggaat

SEQ ID NO: 87 - DNA, 21 bp, synthetic construct
  source 1..21: mol_type = other DNA
ctgagacataggtgcctggcg

SEQ ID NO: 88 - DNA, 20 bp, synthetic construct
  source 1..20: mol_type = other DNA
gaactgagctgcctctaccg

SEQ ID NO: 89 - DNA, 20 bp, synthetic construct
  source 1..20: mol_type = other DNA
gggacaaccctaacacgacc